European Patent Application EP 4 516 310 A1, published March 5, 2025. Title: Lytic agent for Enterococcus faecalis. Applicant: The University of Tokyo. Application JP. The sequence listing filed with the application follows.

SEQUENCE LISTING (12 sequences)

SEQ ID NO: 1 - protein, 330 aa, Enterococcus faecalis-derived prophage
MTLNGIDISSWQSNINVGKEGVSADFVIIKATGGTGYINPDCDRAFQQAISSGKKVAVYHFANEVGLEGTAEQEAEFFLKNIKGYIGKAVLVLDWESTNKGDVPWAKRWLDYVQSKTGVKPMFYTYTNVLQSYNFSSIAKADYGLWLADYGANNPQGYSQPTPPSVPYWNFISMYQYTSNGQLPGWNGRLDLNVFFGDRNMWDKYANPKSNPTPAPPVPPKPKRRYGYRVDDLQFVNGIWQVRNDVLGQPDFDWTENGINVAYIDKINPATGENTPDQELKVGDYFAFQPSSVGIITEQYSLNGKTISHVQFPDEFIWLYTESVEKLIYG

SEQ ID NO: 2 - DNA, 993 bp, Enterococcus faecalis-derived prophage
  source 1..993: mol_type = unassigned DNA
atgacattaaacggaattgatatttctagttggcaatcaaatattaatgtaggtaaagaaggggtttctgcggattttgttattattaaagcaacaggtggaacaggatatataaatcctgactgtgatagagcattccaacaagcaattagtagtggtaaaaaagtagctgtatatcattttgcaaatgaagtaggacttgaagggacagcggagcaagaagctgagttctttttaaaaaatattaaaggttatatcggtaaggccgtcttggttttagactgggaaagtactaataaaggggacgttccttgggctaaacgttggttagattatgttcaaagtaaaacaggggtaaaacctatgttttatacttataccaatgttttacaatcatataattttagctctattgcaaaagctgattatggtttgtggttagctgattacggagcaaataatccacaaggatattcccaaccaactccgccatcagttccttattggaattttatttcaatgtatcaatatacctcaaatggtcaattgcctggctggaatggtcgattagatttaaatgtattctttggtgatagaaacatgtgggacaaatacgctaatcccaaaagtaatccgacacccgctcctccagttcctcctaaacctaagcgccgttacggatatagagtagacgatttacaatttgtaaacggtatttggcaagtaagaaatgatgtattggggcagccggactttgattggacagaaaacggaattaatgttgcttatattgataagatcaatccagcaacaggagagaatactccagatcaagaattaaaagtcggagactattttgcttttcaaccatcttctgtagggattattactgaacaatactctttaaatgggaaaacaatctcgcatgttcaattcccagatgaatttatttggttgtacacagaaagtgttgagaaattaatctatgggtaa

SEQ ID NO: 3 - DNA, 37 bp, synthetic construct
  misc_feature 29: note = a, c, g, or t
  source 1..37: mol_type = other DNA
acacgacgctcttccgatctcctacgggnggcwgcag

SEQ ID NO: 4 - DNA, 41 bp, synthetic construct
  source 1..41: mol_type = other DNA
gacgtgtgctcttccgatctgactachvgggtatctaatcc

SEQ ID NO: 5 - DNA, 20 bp, synthetic construct
  source 1..20: mol_type = other DNA
acacgacgctcttccgatct

SEQ ID NO: 6 - DNA, 20 bp, synthetic construct
  source 1..20: mol_type = other DNA
gacgtgtgctcttccgatct

SEQ ID NO: 7 - DNA, 12 bp, synthetic construct
  source 1..12: mol_type = other DNA
atcaagtagtct

SEQ ID NO: 8 - DNA, 18 bp, synthetic construct
  source 1..18: mol_type = other DNA
acgattcaaagctaactg

SEQ ID NO: 9 - DNA, 21 bp, synthetic construct
  source 1..21: mol_type = other DNA
ttgaggcagaccagattgacg

SEQ ID NO: 10 - DNA, 21 bp, synthetic construct
  source 1..21: mol_type = other DNA
tatgacagcgactccgattcc

SEQ ID NO: 11 - DNA, 28 bp, synthetic construct
  source 1..28: mol_type = other DNA
aaggatccatgacattaaacggaattga

SEQ ID NO: 12 - DNA, 28 bp, synthetic construct
  source 1..28: mol_type = other DNA
aagtcgacttacccatagattaatttct